European Patent Application EP 4 789 727 A1, published August 12, 2026. Title: ANTIBODY FOR USE IN A THERAPY OF AN IgE-ASSOCIATED DISEASE. Applicant: UNIVERSITÄTSKLINIKUM HAMBURG-EPPENDORF (UKE). Application EP. The sequence listing filed with the application follows.

SEQUENCE LISTING (41 sequences)

SEQ ID NO: 1 - protein, 52 aa, synthetic construct
  VARIANT 16: note = x = V or L
GLAGGSAQSQRAPDRXLCHSGQQQGLPRAAGGSVPHPRCHCGAGRADWPGPP

SEQ ID NO: 2 - protein, 12 aa, synthetic construct
QSLLYSSNQKNY

SEQ ID NO: 3 - protein, 9 aa, synthetic construct
QQYYSYPWT

SEQ ID NO: 4 - protein, 9 aa, synthetic construct
GYSITSGYY

SEQ ID NO: 5 - protein, 7 aa, synthetic construct
ISYDGSN

SEQ ID NO: 6 - protein, 9 aa, synthetic construct
ARDYGGFDY

SEQ ID NO: 7 - protein, 248 aa, synthetic construct
  REGION 27..38: note = LCDR1
  REGION 56..58: note = LCDR2
  REGION 95..103: note = LCDR3
  REGION 155..163: note = HCDR1
  REGION 181..187: note = HCDR2
  REGION 226..234: note = HCDR3
  REGION 115..129: note = Whitlow-Linker
DIVMSQSPSSLAVSVGEKVTMSCKSSQSLLYSSNQKNYLAWYQQKPGQSPKLLIYWASTRESGVPDRFTGSGSGTDFTLTISSVKAEDLAVYYCQQYYSYPWTFGGGTKLEIKRGSTSGSGKPGSGEGSDVQLQESGPGLVKPSQSLSLTCSVTGYSITSGYYWNWIRQFPGNKLEWMGSISYDGSNNYNPSLKNRISITRDTSKNQFFLKLNSVTTEDTATYYCARDYGGFDYWGQGTTLTVSSAAA

SEQ ID NO: 8 - protein, 5 aa, synthetic construct
RYTMH

SEQ ID NO: 9 - protein, 17 aa, synthetic construct
YINPSRGYTNYNQKFKD

SEQ ID NO: 10 - protein, 10 aa, synthetic construct
YYDDHYCLDY

SEQ ID NO: 11 - protein, 10 aa, synthetic construct
RASSSVSYMN

SEQ ID NO: 12 - protein, 7 aa, synthetic construct
DTSKVAS

SEQ ID NO: 13 - protein, 9 aa, synthetic construct
QQWSSNPLT

SEQ ID NO: 14 - protein, 243 aa, synthetic construct
  REGION 31..35: note = HCDR1
  REGION 50..66: note = HCDR2
  REGION 99..108: note = HCDR3
  REGION 122..135: note = GS-Linker
  REGION 161..170: note = LCDR1
  REGION 186..192: note = LCDR2
  REGION 225..233: note = LCDR3
DIKLQQSGAELARPGASVKMSCKTSGYTFTRYTMHWVKQRPGQGLEWIGYINPSRGYTNYNQKFKDKATLTTDKSSSTAYMQLSSLTSEDSAVYYCARYYDDHYCLDYWGQGTTLTVSSVEGGSGGSGGSGGSGGVDDIQLTQSPAIMSASPGEKVTMTCRASSSVSYMNWYQQKSGTSPKRWIYDTSKVASGVPYRFSGSGSGTSYSLTISSMEAEDAATYYCQQWSSNPLTFGAGTKLELK

SEQ ID NO: 15 - protein, 5 aa, synthetic construct
DYGMS

SEQ ID NO: 16 - protein, 17 aa, synthetic construct
DISWNGGSTYYADSVKG

SEQ ID NO: 17 - protein, 11 aa, synthetic construct
MGEGGWGANDY

SEQ ID NO: 18 - protein, 120 aa, synthetic construct
  REGION 31..35: note = CDR1
  REGION 50..66: note = CDR2
  REGION 99..109: note = CDR3
EVQLVESGGGLVQPGGSLRLSCAASGFTFDDYGMSWVRQAPGKWLEWVSDISWNGGSTYYADSVKGRFTISRDNAENTLYLQMNSLKPDDTAVYYCAKMGEGGWGANDYWGQGTQVTVSS

SEQ ID NO: 19 - protein, 8 aa, synthetic construct
SGLTFSSY

SEQ ID NO: 20 - protein, 17 aa, synthetic construct
REFVASITWSGRDTFYA

SEQ ID NO: 21 - protein, 11 aa, synthetic construct
PWPVAAPRSGT

SEQ ID NO: 22 - protein, 122 aa, synthetic construct
  VARIANT 14: note = X = A or P
  REGION 25..32: note = CDR1
  REGION 45..61: note = CDR2
  REGION 99..110: note = CDR3
EVQLVESGGELVQXGGSLRLSCAASGLTFSSYNMGWFRRAPGKEREFVASITWSGRDTFYADSVKGRFTISRDNAKNTVYLQMSSLKPEDTAVYYCAANPWPVAAPRSGTYWGQGTQVTVSS

SEQ ID NO: 23 - protein, 15 aa, synthetic construct
MGWSCIILFLVATAT

SEQ ID NO: 24 - protein, 7 aa, synthetic construct
SSGGGGS

SEQ ID NO: 25 - protein, 6 aa, synthetic construct
GSGGGS

SEQ ID NO: 26 - protein, 9 aa, synthetic construct
GGGGSGGGS

SEQ ID NO: 27 - protein, 11 aa, synthetic construct
SSGGGGSGGGS

SEQ ID NO: 28 - protein, 14 aa, synthetic construct
GGSGGSGGSGGSGG

SEQ ID NO: 29 - protein, 15 aa, synthetic construct
GSTSGSGKPGSGEGS

SEQ ID NO: 30 - protein, 18 aa, synthetic construct
GSTSGSGKPGSGEGSTKG

SEQ ID NO: 31 - protein, 115 aa, synthetic construct
  VARIANT 87: note = X = R or A
EVQLVESGGGLVQPGNSLRLSCAASGFTFSSFGMSWVRQAPGKGLEWVSSISGSGSDTLYADSVKGRFTISRDNAKTTLYLQMNSLXPEDTAVYYCTIGGSLSRSSQGTLVTVSS

SEQ ID NO: 32 - DNA, 1578 bp, synthetic construct
  source 1..1578: mol_type = other DNA
atgggatggagctgtatcatcctcttcttggtagcaacagctacaggcgcgcactccatggccgatatcgttatgtctcaatcaccgtcttctctggcggtctccgtgggtgaaaaggtgacgatgtcctgtaaaagttcacaatctctgttgtactcaagtaaccagaagaattatctcgcatggtatcaacaaaagcctggacaatccccaaagttgctcatctattgggccagtacccgagagagcggcgtgccagatcggtttactggatcaggctccggtactgactttaccctgacaatttccagcgttaaagccgaggatctcgccgtctactattgccaacagtactactcctacccttggacttttggtggcggaacaaaactcgagattaagcgaggatccacgtcaggctccggcaaaccaggctccggcgaaggatcagacgttcaattgcaagaatccggccccggactggtaaagccaagccaaagtcttagcctgacttgttcagtgacgggatatagcattacttctgggtactattggaattggattcgccaattccccggaaataagttggagtggatgggatctatttcatatgatggcagtaacaattataaccccagcctgaagaacagaataagcattacccgcgatactagtaagaatcaattctttcttaaactcaactcagtcacaaccgaagatacggcaacttactattgcgcccgagattatggcgggttcgattattggggccaggggactaccttgaccgtgagtagcgcggccgcttcttctggtggcggcggaagcgatatcaagctccagcaatctggcgccgagctggctagacctggcgcctctgtgaagatgagctgcaagaccagcggctacaccttcaccagatacaccatgcactgggtcaagcagaggccaggccaaggcttggagtggatcggctacatcaaccccagccggggctacaccaactacaaccagaagttcaaggacaaggccacactgaccaccgacaagagcagcagcacagcctacatgcagctgagcagcctgaccagcgaagatagcgccgtgtactactgcgcccggtactacgacgatcactactgcctggattactggggccagggcacaaccctgacagtgtcatctgtggaaggcggctctggtggcagtggtggaagcggaggatctggcggagtggacgatatccagctgacacagagccccgccatcatgagtgctagccctggcgagaaagtgaccatgacctgtagagccagcagcagcgtgtcctacatgaactggtatcagcagaagtccggcacaagccccaagcggtggatctacgatacaagcaaggtggccagcggcgtgccctacagattttctggctctggcagcggcaccagctactccctgacaatcagcagcatggaagccgaggacgccgccacttactactgccagcagtggtctagcaaccctctgacctttggagccggcaccaagctggaactgaagcaccaccaccatcaccactaa

SEQ ID NO: 33 - protein, 525 aa, synthetic construct
  REGION 1..15: note = IgH signal domain
  REGION 22..269: note = scFv 2E3E10 domain
  REGION 270..276: note = GS linker
  REGION 277..519: note = Blinatumomab anti-CD3 scFv domain
  REGION 520..525: note = His tag
MGWSCIILFLVATATGAHSMADIVMSQSPSSLAVSVGEKVTMSCKSSQSLLYSSNQKNYLAWYQQKPGQSPKLLIYWASTRESGVPDRFTGSGSGTDFTLTISSVKAEDLAVYYCQQYYSYPWTFGGGTKLEIKRGSTSGSGKPGSGEGSDVQLQESGPGLVKPSQSLSLTCSVTGYSITSGYYWNWIRQFPGNKLEWMGSISYDGSNNYNPSLKNRISITRDTSKNQFFLKLNSVTTEDTATYYCARDYGGFDYWGQGTTLTVSSAAASSGGGGSDIKLQQSGAELARPGASVKMSCKTSGYTFTRYTMHWVKQRPGQGLEWIGYINPSRGYTNYNQKFKDKATLTTDKSSSTAYMQLSSLTSEDSAVYYCARYYDDHYCLDYWGQGTTLTVSSVEGGSGGSGGSGGSGGVDDIQLTQSPAIMSASPGEKVTMTCRASSSVSYMNWYQQKSGTSPKRWIYDTSKVASGVPYRFSGSGSGTSYSLTISSMEAEDAATYYCQQWSSNPLTFGAGTKLELKHHHHHH

SEQ ID NO: 34 - DNA, 1923 bp, synthetic construct
  source 1..1923: mol_type = other DNA
atgggatggagctgtatcatcctcttcttggtagcaacagctacaggcgcgcactccatggccgatatcgttatgtctcaatcaccgtcttctctggcggtctccgtgggtgaaaaggtgacgatgtcctgtaaaagttcacaatctctgttgtactcaagtaaccagaagaattatctcgcatggtatcaacaaaagcctggacaatccccaaagttgctcatctattgggccagtacccgagagagcggcgtgccagatcggtttactggatcaggctccggtactgactttaccctgacaatttccagcgttaaagccgaggatctcgccgtctactattgccaacagtactactcctacccttggacttttggtggcggaacaaaactcgagattaagcgaggatccacgtcaggctccggcaaaccaggctccggcgaaggatcagacgttcaattgcaagaatccggccccggactggtaaagccaagccaaagtcttagcctgacttgttcagtgacgggatatagcattacttctgggtactattggaattggattcgccaattccccggaaataagttggagtggatgggatctatttcatatgatggcagtaacaattataaccccagcctgaagaacagaataagcattacccgcgatactagtaagaatcaattctttcttaaactcaactcagtcacaaccgaagatacggcaacttactattgcgcccgagattatggcgggttcgattattggggccaggggactaccttgaccgtgagtagcgcggccgcttcttctggtggcggcggaagcgatatcaagctccagcaatctggcgccgagctggctagacctggcgcctctgtgaagatgagctgcaagaccagcggctacaccttcaccagatacaccatgcactgggtcaagcagaggccaggccaaggcttggagtggatcggctacatcaaccccagccggggctacaccaactacaaccagaagttcaaggacaaggccacactgaccaccgacaagagcagcagcacagcctacatgcagctgagcagcctgaccagcgaagatagcgccgtgtactactgcgcccggtactacgacgatcactactgcctggattactggggccagggcacaaccctgacagtgtcatctgtggaaggcggctctggtggcagtggtggaagcggaggatctggcggagtggacgatatccagctgacacagagccccgccatcatgagtgctagccctggcgagaaagtgaccatgacctgtagagccagcagcagcgtgtcctacatgaactggtatcagcagaagtccggcacaagccccaagcggtggatctacgatacaagcaaggtggccagcggcgtgccctacagattttctggctctggcagcggcaccagctactccctgacaatcagcagcatggaagccgaggacgccgccacttactactgccagcagtggtctagcaaccctctgacctttggagccggcaccaagctggaactgaagggatccggcggtggaagcgaggtccaacttgtagaatctgggggcggtctcgtccaacccggaaattcattgcgcctttcatgcgcagccagtgggtttactttcagttccttcgggatgtcatgggtaagacaagcaccaggtaaaggcttggagtgggtgtccagtatctctggctctggaagcgatacactttacgcggattccgtgaaaggacggtttacaatttcacgggataacgctaaaacaacattgtatctgcaaatgaactcacttcgacccgaggatacggcagtgtattattgtacaatagggggatcattgagtcgatcctcacaaggcaccctcgttacagtaagctcctaa

SEQ ID NO: 35 - protein, 640 aa, synthetic construct
  REGION 1..15: note = IgH signal domain
  REGION 22..269: note = scFv 2E3E10 domain
  REGION 270..276: note = GS linker
  REGION 277..519: note = Blinatumomab anti-CD3 domain
  REGION 520..525: note = GS linker
  REGION 526..640: note = anti-HSA domain
MGWSCIILFLVATATGAHSMADIVMSQSPSSLAVSVGEKVTMSCKSSQSLLYSSNQKNYLAWYQQKPGQSPKLLIYWASTRESGVPDRFTGSGSGTDFTLTISSVKAEDLAVYYCQQYYSYPWTFGGGTKLEIKRGSTSGSGKPGSGEGSDVQLQESGPGLVKPSQSLSLTCSVTGYSITSGYYWNWIRQFPGNKLEWMGSISYDGSNNYNPSLKNRISITRDTSKNQFFLKLNSVTTEDTATYYCARDYGGFDYWGQGTTLTVSSAAASSGGGGSDIKLQQSGAELARPGASVKMSCKTSGYTFTRYTMHWVKQRPGQGLEWIGYINPSRGYTNYNQKFKDKATLTTDKSSSTAYMQLSSLTSEDSAVYYCARYYDDHYCLDYWGQGTTLTVSSVEGGSGGSGGSGGSGGVDDIQLTQSPAIMSASPGEKVTMTCRASSSVSYMNWYQQKSGTSPKRWIYDTSKVASGVPYRFSGSGSGTSYSLTISSMEAEDAATYYCQQWSSNPLTFGAGTKLELKGSGGGSEVQLVESGGGLVQPGNSLRLSCAASGFTFSSFGMSWVRQAPGKGLEWVSSISGSGSDTLYADSVKGRFTISRDNAKTTLYLQMNSLRPEDTAVYYCTIGGSLSRSSQGTLVTVSS

SEQ ID NO: 36 - DNA, 1575 bp, synthetic construct
  source 1..1575: mol_type = other DNA
atgggatggagctgtatcatcctcttcttggtagcaacagctacaggcgcgcactccatggccgatatcgttatgtctcaatcaccgtcttctctggcggtctccgtgggtgaaaaggtgacgatgtcctgtaaaagttcacaatctctgttgtactcaagtaaccagaagaattatctcgcatggtatcaacaaaagcctggacaatccccaaagttgctcatctattgggccagtacccgagagagcggcgtgccagatcggtttactggatcaggctccggtactgactttaccctgacaatttccagcgttaaagccgaggatctcgccgtctactattgccaacagtactactcctacccttggacttttggtggcggaacaaaactcgagattaagcgaggatccacgtcaggctccggcaaaccaggctccggcgaaggatcagacgttcaattgcaagaatccggccccggactggtaaagccaagccaaagtcttagcctgacttgttcagtgacgggatatagcattacttctgggtactattggaattggattcgccaattccccggaaataagttggagtggatgggatctatttcatatgatggcagtaacaattataaccccagcctgaagaacagaataagcattacccgcgatactagtaagaatcaattctttcttaaactcaactcagtcacaaccgaagatacggcaacttactattgcgcccgagattatggcgggttcgattattggggccaggggactaccttgaccgtgagtagcgcggccgctggaggagggggatcaggaggcgggagcgaagtgcagttggtcgagtcagggggcgagctggtgcaacccggtggttcactccggctttcctgtgccgcctctggtctgacttttagctcttataacatggggtggttcaggcgagcgcccggtaaggagcgggagttcgtcgcatctatcacctggtcaggtcgggacaccttttacgcggacagtgtgaaaggacgatttacaatctcaagggataatgcaaagaatacggtttacttgcaaatgtctagcttgaagcctgaggacactgccgtctactattgcgccgctaatccctggccagtggctgcgccgcggagtggcacttattgggggcaaggtacccaggtcaccgtgagttctggcggagggggatccggcggtggaagcgaggtccaacttgtagaatctgggggcggtctcgtccaacccggaaattcattgcgcctttcatgcgcagccagtgggtttactttcagttccttcgggatgtcatgggtaagacaagcaccaggtaaaggcttggagtgggtgtccagtatctctggctctggaagcgatacactttacgcggattccgtgaaaggacggtttacaatttcacgggataacgctaaaacaacattgtatctgcaaatgaactcacttcgacccgaggatacggcagtgtattattgtacaatagggggatcattgagtcgatcctcacaaggcaccctcgttacagtaagctcctaa

SEQ ID NO: 37 - protein, 524 aa, synthetic construct
  REGION 1..15: note = IgH signal domain
  REGION 22..269: note = scFv 2E3E10 domain
  REGION 270..278: note = GS linker
  REGION 279..398: note = anti-CD16 nanobody c21
  REGION 399..409: note = GS linker
  REGION 410..524: note = anti-HSA domain
MGWSCIILFLVATATGAHSMADIVMSQSPSSLAVSVGEKVTMSCKSSQSLLYSSNQKNYLAWYQQKPGQSPKLLIYWASTRESGVPDRFTGSGSGTDFTLTISSVKAEDLAVYYCQQYYSYPWTFGGGTKLEIKRGSTSGSGKPGSGEGSDVQLQESGPGLVKPSQSLSLTCSVTGYSITSGYYWNWIRQFPGNKLEWMGSISYDGSNNYNPSLKNRISITRDTSKNQFFLKLNSVTTEDTATYYCARDYGGFDYWGQGTTLTVSSAAAGGGGSGGGSEVQLVESGGELVQPGGSLRLSCAASGLTFSSYNMGWFRRAPGKEREFVASITWSGRDTFYADSVKGRFTISRDNAKNTVYLQMSSLKPEDTAVYYCAANPWPVAAPRSGTYWGQGTQVTVSSGGGGSGGGSEVQLVESGGGLVQPGNSLRLSCAASGFTFSSFGMSWVRQAPGKGLEWVSSISGSGSDTLYADSVKGRFTISRDNAKTTLYLQMNSLRPEDTAVYYCTIGGSLSRSSQGTLVTVSS

SEQ ID NO: 38 - DNA, 1194 bp, synthetic construct
  source 1..1194: mol_type = other DNA
atgggatggagctgtatcatcctcttcttggtagcaacagctacaggcgcgcactccatggccgatatcgttatgtctcaatcaccgtcttctctggcggtctccgtgggtgaaaaggtgacgatgtcctgtaaaagttcacaatctctgttgtactcaagtaaccagaagaattatctcgcatggtatcaacaaaagcctggacaatccccaaagttgctcatctattgggccagtacccgagagagcggcgtgccagatcggtttactggatcaggctccggtactgactttaccctgacaatttccagcgttaaagccgaggatctcgccgtctactattgccaacagtactactcctacccttggacttttggtggcggaacaaaactcgagattaagcgaggatccacgtcaggctccggcaaaccaggctccggcgaaggatcagacgttcaattgcaagaatccggccccggactggtaaagccaagccaaagtcttagcctgacttgttcagtgacgggatatagcattacttctgggtactattggaattggattcgccaattccccggaaataagttggagtggatgggatctatttcatatgatggcagtaacaattataaccccagcctgaagaacagaataagcattacccgcgatactagtaagaatcaattctttcttaaactcaactcagtcacaaccgaagatacggcaacttactattgcgcccgagattatggcgggttcgattattggggccaggggactaccttgaccgtgagtagcgcggccgctgaggtgcaacttgtcgaaagtggggggggattagtgcagcctggcgggtctctccggctgtcatgtgcggcttctggctttacgttcgatgattatgggatgtcctgggtccgccaagcgccaggaaagtggctggagtgggtttctgacatttcttggaacggcggctcaacttattacgctgattccgttaaagggcggtttaccattagcagggacaatgcagagaacacactttatcttcaaatgaatagcttgaaacccgatgatacggccgtgtattattgcgctaaaatgggagagggtggctggggtgcaaacgattattggggtcaaggcacacaggtgacagtaagtagcggatcccaccatcatcaccatcattaa

SEQ ID NO: 39 - protein, 397 aa, synthetic construct
  REGION 1..15: note = IgH signal domain
  REGION 22..269: note = scFv 2E3E10 domain
  REGION 270..389: note = anti-CD3 nanobody 3D-H11
  REGION 390..391: note = GS linker
  REGION 392..397: note = His tag
MGWSCIILFLVATATGAHSMADIVMSQSPSSLAVSVGEKVTMSCKSSQSLLYSSNQKNYLAWYQQKPGQSPKLLIYWASTRESGVPDRFTGSGSGTDFTLTISSVKAEDLAVYYCQQYYSYPWTFGGGTKLEIKRGSTSGSGKPGSGEGSDVQLQESGPGLVKPSQSLSLTCSVTGYSITSGYYWNWIRQFPGNKLEWMGSISYDGSNNYNPSLKNRISITRDTSKNQFFLKLNSVTTEDTATYYCARDYGGFDYWGQGTTLTVSSAAAEVQLVESGGGLVQPGGSLRLSCAASGFTFDDYGMSWVRQAPGKWLEWVSDISWNGGSTYYADSVKGRFTISRDNAENTLYLQMNSLKPDDTAVYYCAKMGEGGWGANDYWGQGTQVTVSSGSHHHHHH

SEQ ID NO: 40 - DNA, 1533 bp, synthetic construct
  source 1..1533: mol_type = other DNA
atgggatggagctgtatcatcctcttcttggtagcaacagctacaggcgcgcactccatggccgatatcgttatgtctcaatcaccgtcttctctggcggtctccgtgggtgaaaaggtgacgatgtcctgtaaaagttcacaatctctgttgtactcaagtaaccagaagaattatctcgcatggtatcaacaaaagcctggacaatccccaaagttgctcatctattgggccagtacccgagagagcggcgtgccagatcggtttactggatcaggctccggtactgactttaccctgacaatttccagcgttaaagccgaggatctcgccgtctactattgccaacagtactactcctacccttggacttttggtggcggaacaaaactcgagattaagcgaggatccacgtcaggctccggcaaaccaggctccggcgaaggatcagacgttcaattgcaagaatccggccccggactggtaaagccaagccaaagtcttagcctgacttgttcagtgacgggatatagcattacttctgggtactattggaattggattcgccaattccccggaaataagttggagtggatgggatctatttcatatgatggcagtaacaattataaccccagcctgaagaacagaataagcattacccgcgatactagtaagaatcaattctttcttaaactcaactcagtcacaaccgaagatacggcaacttactattgcgcccgagattatggcgggttcgattattggggccaggggactaccttgaccgtgagtagcgcggccgctgaggtgcaacttgtcgaaagtggggggggattagtgcagcctggcgggtctctccggctgtcatgtgcggcttctggctttacgttcgatgattatgggatgtcctgggtccgccaagcgccaggaaagtggctggagtgggtttctgacatttcttggaacggcggctcaacttattacgctgattccgttaaagggcggtttaccattagcagggacaatgcagagaacacactttatcttcaaatgaatagcttgaaacccgatgatacggccgtgtattattgcgctaaaatgggagagggtggctggggtgcaaacgattattggggtcaaggcacacaggtgacagtaagtagcggatccggcggtggaagcgaggtccaacttgtagaatctgggggcggtctcgtccaacccggaaattcattgcgcctttcatgcgcagccagtgggtttactttcagttccttcgggatgtcatgggtaagacaagcaccaggtaaaggcttggagtgggtgtccagtatctctggctctggaagcgatacactttacgcggattccgtgaaaggacggtttacaatttcacgggataacgctaaaacaacattgtatctgcaaatgaactcacttcgacccgaggatacggcagtgtattattgtacaatagggggatcattgagtcgatcctcacaaggcaccctcgttacagtaagctcctaa

SEQ ID NO: 41 - protein, 510 aa, synthetic construct
  REGION 1..15: note = IgH signal domain
  REGION 22..269: note = scFv 2E3E10 domain
  REGION 270..389: note = anti-CD3 nanobody 3D-H11
  REGION 390..395: note = GS linker
  REGION 396..510: note = anti HSA domain
MGWSCIILFLVATATGAHSMADIVMSQSPSSLAVSVGEKVTMSCKSSQSLLYSSNQKNYLAWYQQKPGQSPKLLIYWASTRESGVPDRFTGSGSGTDFTLTISSVKAEDLAVYYCQQYYSYPWTFGGGTKLEIKRGSTSGSGKPGSGEGSDVQLQESGPGLVKPSQSLSLTCSVTGYSITSGYYWNWIRQFPGNKLEWMGSISYDGSNNYNPSLKNRISITRDTSKNQFFLKLNSVTTEDTATYYCARDYGGFDYWGQGTTLTVSSAAAEVQLVESGGGLVQPGGSLRLSCAASGFTFDDYGMSWVRQAPGKWLEWVSDISWNGGSTYYADSVKGRFTISRDNAENTLYLQMNSLKPDDTAVYYCAKMGEGGWGANDYWGQGTQVTVSSGSGGGSEVQLVESGGGLVQPGNSLRLSCAASGFTFSSFGMSWVRQAPGKGLEWVSSISGSGSDTLYADSVKGRFTISRDNAKTTLYLQMNSLRPEDTAVYYCTIGGSLSRSSQGTLVTVSS